European Patent Specification EP 3 612 189 B1, published September 27, 2023. Title: Virus Like Particle. Applicant: The University of York University of Leeds. The sequence listing filed with the application follows.

SEQUENCE LISTING (72 sequences)

SEQ ID NO: 1 - RNA, 35 nt, artificial sequence
  Packaging signal
guuuguuuaaagacugggaggaguugggggaggag

SEQ ID NO: 2 - RNA, 49 nt, artificial sequence
  Packaging signal
gggcccucugacaguuaaugaaaaaaggagauuaaaauuaauuaugccu

SEQ ID NO: 3 - RNA, 34 nt, artificial sequence
  Packaging signal
ggcuggcauucuauauaagagagaaacuacacgc

SEQ ID NO: 4 - RNA, 59 nt, artificial sequence
  Packaging signal
cugggaggaguugggggaggagauuagguuaaaggucuuuguacuaggaggcuguaggc

SEQ ID NO: 5 - RNA, 135 nt, artificial sequence
  Packaging signal
gggcugcccucaaggaccagggcagaaaagaggaaaagaaaagugacagaacacuuauaaggaaaaaacguacaaacguuuuaaggaaaaaaggaagcugcaauagcgcaaggaauccgaaaauucggaaaggaa

SEQ ID NO: 6 - RNA, 129 nt, artificial sequence
  Packaging signal
gggcugcccucaaggaccagggcagaaaagaggaaaagaaaagugacagaacacuuauaaggaaccacacaaguggaaggaaaaaaggaagcugcaauagcgcaaggaauccgaaaauucggaaaggaa

SEQ ID NO: 7 - RNA, 129 nt, artificial sequence
  Packaging signal
gggcugcccucaaggaccagggcagaaaagaggaaaagaaaagugacagaacacuuauaaggaaccacacaaguauaaggaaaaaaggaagcugcaauagcgcaaggaauccgaaaauucggaaaggaa

SEQ ID NO: 8 - RNA, 140 nt, artificial sequence
  Packaging signal
gggccccgcaacaaugcggggaaggaaggaaggaagaaaacguacaaacguuuuaaggaacaacgcaacaaugcguugaaggaaggaaggaaggggcguacaaacgccccaaggaauuuugcaacaaugcaaaaaaggaa

SEQ ID NO: 9 - RNA, 11 nt, artificial sequence
  nucleotide binding motif
gaaaaaaggag

SEQ ID NO: 10 - RNA, 18 nt, artificial sequence
  B3 sequence variants
acaugcaacaaugcacac

SEQ ID NO: 11 - RNA, 18 nt, artificial sequence
  B3 sequence variants
acaugcaauuuugcacac

SEQ ID NO: 12 - RNA, 18 nt, artificial sequence
  B3 sequence variants
acaugcauuuaugcacac

SEQ ID NO: 13 - RNA, 18 nt, artificial sequence
  B3 sequence variants
acaugcaguuuugcacac

SEQ ID NO: 14 - RNA, 18 nt, artificial sequence
  B3 sequence variants
acaugcauuugugcacac

SEQ ID NO: 15 - RNA, 18 nt, artificial sequence
  B3 sequence variants
acaugcaauugugcacac

SEQ ID NO: 16 - RNA, 18 nt, artificial sequence
  B3 sequence variants
acaugcaguuaugcacac

SEQ ID NO: 17 - RNA, 18 nt, artificial sequence
  B3 sequence variants
acaugcaguugugcacac

SEQ ID NO: 18 - RNA, 18 nt, artificial sequence
  B3 sequence variants
acaugcaauuaugcacac

SEQ ID NO: 19 - DNA, 32 bp, artificial sequence
  Primer
gacattaatacgactcactatagggacatgca

SEQ ID NO: 20 - DNA, 33 bp, artificial sequence
  Primer
gtgtgcataattgcatgtccctatagtgagtcg

SEQ ID NO: 21 - DNA, 33 bp, artificial sequence
  Primer
gtgtgcacaactgcatgtccctatagtgagtcg

SEQ ID NO: 22 - DNA, 33 bp, artificial sequence
  Primer
gtgtgcacaattgcatgtccctatagtgagtcg

SEQ ID NO: 23 - DNA, 33 bp, artificial sequence
  Primer
gtgtgcataactgcatgtccctatagtgagtcg

SEQ ID NO: 24 - DNA, 33 bp, artificial sequence
  Primer
gtgtgcataaatgcatgtccctatagtgagtcg

SEQ ID NO: 25 - DNA, 33 bp, artificial sequence
  Primer
gtgtgcaaaattgcatgtccctatagtgagtcg

SEQ ID NO: 26 - DNA, 33 bp, artificial sequence
  Primer
gtgtgcaaaactgcatgtccctatagtgagtcg

SEQ ID NO: 27 - DNA, 33 bp, artificial sequence
  Primer
gtgtgcacaaatgcatgtccctatagtgagtcg

SEQ ID NO: 28 - DNA, 33 bp, artificial sequence
  Primer
gtgtgcatggttgcatgtccctatagtgagtcg

SEQ ID NO: 29 - DNA, 33 bp, artificial sequence
  Primer
gtgtgcatttttgcatgtccctatagtgagtcg

SEQ ID NO: 30 - DNA, 33 bp, artificial sequence
  Primer
gtgtgcatccttgcatgtccctatagtgagtcg

SEQ ID NO: 31 - DNA, 33 bp, artificial sequence
  Primer
gtgtgcatcattgcatgtccctatagtgagtcg

SEQ ID NO: 32 - DNA, 33 bp, artificial sequence
  Primer
gtgtgcatacttgcatgtccctatagtgagtcg

SEQ ID NO: 33 - DNA, 62 bp, artificial sequence
  Primer
agtaatacgactcactataggggggctgccctcaaggaccagggcagaaaagaggaaaagaa

SEQ ID NO: 34 - DNA, 89 bp, artificial sequence
  Primer
ggcagaaaagaggaaaagaaaagtgacagaacacttataaggaaatacacaagtataaggaaaaaaggaagctgcaatagcgcaaggaa

SEQ ID NO: 35 - DNA, 41 bp, artificial sequence
  Primer
ttcctttccgaattttcggattccttgcgctattgcagctt

SEQ ID NO: 36 - DNA, 54 bp, artificial sequence
  Primer
gggccccgcaacaatgcggggaaggaaggaaggaagaaaacgtacaaacgtttt

SEQ ID NO: 37 - DNA, 86 bp, artificial sequence
  Primer
agaaaacgtacaaacgttttaaggaacaacgcaacaatgcgttgaaggaaggaaggaaggggcgtacaaacgccccaaggaatttt

SEQ ID NO: 38 - DNA, 45 bp, artificial sequence
  Primer
ttccttttttgcattgttgcaaaattccttggggcgtttgtacgc

SEQ ID NO: 39 - DNA, 89 bp, artificial sequence
  Primer
ggcagaaaagaggaaaagaaaagtgacagaacacttataaggaaccacacaagtggaaggaaaaaaggaagctgcaatagcgcaaggaa

SEQ ID NO: 40 - DNA, 95 bp, artificial sequence
  Primer
ggcagaaaagaggaaaagaaaagtgacagaacacttataaggaaaaaacguacaaacguuuuaaggaaaaaaggaagctgcaatagcgcaaggaa

SEQ ID NO: 41 - DNA, 61 bp, artificial sequence
  Primer
agtaatacgactcactatagggagtaaagacaggaaactttactgactaacatggcaaaac

SEQ ID NO: 42 - DNA, 80 bp, artificial sequence
  Primer
actgactaacatggcaaaacaacagaacaacaggcgaaaatccgcaacaatgcgtgcagtgaagcgcatgataaatacac

SEQ ID NO: 43 - DNA, 45 bp, artificial sequence
  Primer
tcagtgcaaaccttttatgctccaagtgtgtatttatcatgcgct

SEQ ID NO: 44 - DNA, 61 bp, artificial sequence; identical to SEQ ID NO: 41
  Primer

SEQ ID NO: 45 - DNA, 41 bp, artificial sequence
  Primer
actgactaacatggcaaaacaacagaacaacaggcgaaaat

SEQ ID NO: 46 - DNA, 28 bp, artificial sequence
  Primer
cgcattgttgcggattttcgcctgttgt

SEQ ID NO: 47 - DNA, 52 bp, artificial sequence
  Primer
agtaatacgactcactatagggtggcaaaacaacagaacaacaggcgaaaat

SEQ ID NO: 48 - DNA, 57 bp, artificial sequence
  Primer
aacagaacaacaggcgaaaatccgcaacaatgcgtgcagtgaagcgcatgataaata

SEQ ID NO: 49 - DNA, 45 bp, artificial sequence
  Primer
ccaagtgtgtatttatcatgcgcttcactgcacgcattgttgcgg

SEQ ID NO: 50 - DNA, 35 bp, artificial sequence
  Primer
agtaatacgactcactatagggccgcaacaatgcg

SEQ ID NO: 51 - DNA, 39 bp, artificial sequence
  Primer
ccgcaacaatgcgtgcagtgaagcgcatgataaatacac

SEQ ID NO: 52 - DNA, 45 bp, artificial sequence; identical to SEQ ID NO: 43
  Primer

SEQ ID NO: 53 - protein, 56 aa, artificial sequence
  HBV CP
PAYRPPNAPILSTLPETTVVRRRDRGRSPRRRTPSPRRRRSQSPRRRRSQSRESQC

SEQ ID NO: 54 - RNA, 10 nt, artificial sequence
  loop sequences
agguaggagc

SEQ ID NO: 55 - RNA, 47 nt, artificial sequence
  HBV PS-PS1
ggguuuuggguuuguuuaaagacuggaggaguugggggaggagcccc

SEQ ID NO: 56 - RNA, 47 nt, artificial sequence
  HBV PS-PS2
ggguuuuggggugacaguuaaugaaaaaaggagauuaaaauuacccc

SEQ ID NO: 57 - RNA, 47 nt, artificial sequence
  HBV PS-PS3
ggguuuuggggcuggcauucuauauaagagagaaacuacacgccccc

SEQ ID NO: 58 - RNA, 61 nt, artificial sequence
  HBV PS-Epsilon
uguucauguccuacuguucaagccuccaagcugugccuuggguggcuuuggggcauggaca

SEQ ID NO: 59 - protein, 25 aa, artificial sequence
  STNV CP
ELHTNIMRKVARMTASKRRNNQQKA

SEQ ID NO: 60 - RNA, 30 nt, artificial sequence
  B3
ccuuuucaagacaugcaacaaugcacacag

SEQ ID NO: 61 - RNA, 127 nt, artificial sequence
  PS1-5
gaguaaagacaggaaacuuuacugacuaacauggcaaaacaacagaacaacaggcgaaaauccgcaacaaugcgugcagugaagcgcaugauaaauacacacuuggagcauaaaagguuugcacuga

SEQ ID NO: 62 - RNA, 129 nt, artificial sequence; identical to SEQ ID NO: 6
  stable PS3

SEQ ID NO: 63 - RNA, 140 nt, artificial sequence; identical to SEQ ID NO: 8
  all PS3

SEQ ID NO: 64 - RNA, 18 nt, artificial sequence
  inner variants
acaugcaaccaugcacac

SEQ ID NO: 65 - RNA, 18 nt, artificial sequence
  inner variants
acaugcaaaaaugcacac

SEQ ID NO: 66 - RNA, 18 nt, artificial sequence
  inner variants
acaugcaaggaugcacac

SEQ ID NO: 67 - RNA, 18 nt, artificial sequence
  inner variants
acaugcaaugaugcacac

SEQ ID NO: 68 - RNA, 18 nt, artificial sequence
  inner variants
acaugcaaguaugcacac

SEQ ID NO: 69 - RNA, 73 nt, artificial sequence
  PS1-3
aguaaagacaggaaacuuuacugacuaacauggcaaaacaacagaacaacaggcgaaaauccgcaacaaugcg

SEQ ID NO: 70 - RNA, 65 nt, artificial sequence
  PS2-4
aacaacagaacaacaggcgaaaauccgcaacaaugcgugcagugaagcgcaugauaaauacacac

SEQ ID NO: 71 - RNA, 66 nt, artificial sequence
  PS3-5
ccgcaacaaugcgugcagugaagcgcaugauaaauacacacuuggagcauaaaagguuugcacuga

SEQ ID NO: 72 - RNA, 129 nt, artificial sequence; identical to SEQ ID NO: 7
  unstable PS3